European Patent Application EP 4 800 102 A1, published September 2, 2026. Title: Recombinant Attenuated Herpes Simplex Virus Type II Vacccine. Applicant: THE UNIVERSITY OF TOKYO. The sequence listing filed with the application follows.

SEQUENCE LISTING (7 sequences)

SEQ ID NO: 1 - protein, 481 aa, Herpes simplex virus-2
MACRKFCGVYRRPDKRQEASVPPETNTAPAFPASTFYTPAEDAYLAPGPPETIHPSRPPSPGEAARLCQLQEILAQMHSDEDYPIVDAAGAEEEDEADDDAPDDVAYPEDYAEGRFLSMVSAAPLPGASGHPPVPGRAAPPDVRTCDSGKVGATGFTPEELDTMDREALRAISRGCKPPSTLAKLVTGLGFAIHGALIPGSEGCVFDSSHPNYPHRVIVKAGWYASTSHEARLLRRLNHPAILPLLDLHVVSGVTCLVLPKYHCDLYTYLSKRPSPLGHLQITAVSRQLLSAIDYVHCEGIIHRDIKTENIFINTPENICLGDFGAACFVRGCRSSPFHYGIAGTIDTNAPEVLAGDPYTQVIDIWSAGLVIFETAVHTASLFSAPRDPERRPCDNQIARIIRQAQVHVDEFPTHAESRLTAHYRSRAAGNNRPAWTRPAWTRYYKIHTDVEYLICKALTFDAALRPSAAELLRLPLFHPK

SEQ ID NO: 2 - protein, 620 aa, Herpes simplex virus-2
MAAAATPGAKRPADPARDPDSPPKRPRPNSLDLATVFGPRPAPPRPTSPGAPGSHWPQSPPRGQPDGGAPGEKARPASPALSEASSGPPTPDIPLSPGGAHAIDPDCSPGPPDPDPMWSASAIPNALPPHILAETFERHLRGLLRGVRSPLAIGPLWARLDYLCSLVVSLEAAGMVDRGLGRHLWRLTRRAPPSAAEAVAPRPLMGFYEAATQNQADCQLWALLRRGLTTASTLRWGAQGPCFSSQWLTHNASLRLDAQSSAVMFGRVNEPTARNLLFRYCVGRADAGVNDDADAGRFVFHQPGDLAEENVHACGVLMDGHTGMVGASLDILVCPRDPHGYLAPAPQTPLAFYEVKCRAKYAFDPADPGAPAASAYEDLMARRSPEAFRAFIRSIPNPGVRYFAPGRVPGPEEALVTQDRDWLDSRAAGEKRRCSAPDRALVELNSGVVSEVLLFGVPDLERRTISPVAWSSGELVRREPIFANPRHPNFKQILVQGYVLDSHFPDCPLQPHLVTFLGRHRAGAEEGVTFRLEDGRGAPAGRGGAPGPAKASILPDQAVPIALIITPVRVEPGIYRDIRRNSRLAFDDTLAKLWASRSPGRGPAAADTTSSPPTAGRSSR

SEQ ID NO: 3 - protein, 518 aa, Herpes simplex virus-2
MDESGRQRPASHVAADISPQGAHRRSFKAWLASYIHSLSRRASGRPSGPSPRDGAVSGARPGSRRRSSFRERLRAGLSRWRVSRSSRRRSSPEAPGPAAKLRRPPLRRSETAMTSPPSPPSHILSLARIHKLCIPVFAVNPALRYTTLEIPGARSFGGSGGYGEVQLIREHKLAVKTIREKEWFAVELVATLLVGECALRGGRTHDIRGFITPLGFSLQQRQIVFPAYDMDLGKYIGQLASLRATTPSVATALHHCFTDLARAVVFLNTRCGISHLDIKCANVLVMLRSDAVSLRRAVLADFSLVTLNSNSTISRGQFCLQEPDLESPRGFGMPAALTTANFHTLVGHGYNQPPELSVKYLNNERAEFNNRPLKHDVGLAVDLYALGQTLLELLVSVYVAPSLGVPVTRVPGYQYFNNQLSPDFAVALLAYRCVLHPALFVNSAETNTHGLAYDVPEGIRRHLRNPKIRRAFTEQCINYQRTHKAVLSSVSLPPELRPLLVLVSRLCHANPAARHSLS

SEQ ID NO: 4 - protein, 904 aa, Herpes simplex virus-2
MRGGGLICALVVGALVAAVASAAPAAPAAPRASGGVAATVAANGGPASRPPPVPSPATTKARKRKTKKPPKRPEATPPPDANATVAAGHATLRAHLREIKVENADAQFYVCPPPTGATVVQFEQPRRCPTRPEGQNYTEGIAVVFKENIAPYKFKATMYYKDVTVSQVWFGHRYSQFMGIFEDRAPVPFEEVIDKINAKGVCRSTAKYVRNNMETTAFHRDDHETDMELKPAKVATRTSRGWHTTDLKYNPSRVEAFHRYGTTVNCIVEEVDARSVYPYDEFVLATGDFVYMSPFYGYREGSHTEHTSYAADRFKQVDGFYARDLTTKARATSPTTRNLLTTPKFTVAWDWVPKRPAVCTMTKWQEVDEMLRAEYGGSFRFSSDAISTTFTTNLTEYSLSRVDLGDCIGRDAREAIDRMFARKYNATHIKVGQPQYYLATGGFLIAYQPLLSNTLAELYVREYMREQDRKPRNATPAPLREAPSANASVERIKTTSSIEFARLQFTYNHIQRHVNDMLGRIAVAWCELQNHELTLWNEARKLNPNAIASATVGRRVSARMLGDVMAVSTCVPVAPDNVIVQNSMRVSSRPGTCYSRPLVSFRYEDQGPLIEGQLGENNELRLTRDALEPCTVGHRRYFIFGGGYVYFEEYAYSHQLSRADVTTVSTFIDLNITMLEDHEFVPLEVYTRHEIKDSGLLDYTEVQRRNQLHDLRFADIDTVIRADANAAMFAGLCAFFEGMGDLGRAVGKVVMGVVGGVVSAVSGVSSFMSNPFGALAVGLLVLAGLVAAFFAFRYVLQLQRNPMKALYPLTTKELKTSDPGGVGGEGEEGAEGGGFDEAKLAEAREMIRYMALVSAMERTEHKARKKGTSALLSSKVTNMVLRKRNKARYSPLHNEDEAGDEDEL

SEQ ID NO: 5 - protein, 112 aa, Herpes simplex virus-2
MAAPQFHRPSTITADNVRALGMRGLVLATNNAQFIMDNSYPHPHGTQGAVREFLRGQAAALTDLGVTHANNTFAPQPMFAGDAAAEWLRPSFGLKRTYSPFVVRDPKTPSTP

SEQ ID NO: 6 - protein, 492 aa, Herpes simplex virus-2
MGLFGMMKFAQTHHLVKRRGLRAPEGYFTPIAVDLWNVMYTLVVKYQRRYPSYDREAITLHCLCSMLRVFTQKSLFPIFVTDRGVECTEPVVFGAKAILARTTAQCRTDEEASDVDASPPPSPITDSRPSFAFSNMRRRGHAFAPGDRGTRAAGPGPAAPSGAPSKPALRLAHLFCIRVLRALGYAYINSGQLEADDACANLYHTNTVAYVHTTDTDLLLMGCDIVLDISTGYIPTIHCRDLLQYFKMSYPQFLALFVRCHTDLHPNNTYASVEDVLRECHWTAPSRSQARRAARRERANSRSLESMPTLTAAPVGLETRISWTEILAQQIAGEDDYEEDPPLQPPDVAGGPRDGARSSSSEILTPPELVQVPNAQRVAEHRGYVAGRRRHVIHDAPEALDWLPDPMTIAELVEHRYVKYVISLISPKERGPWTLLKRLPIYQDLRDEDLARSIVTRHITAPDIADRFLAQLWAHAPPPAFYKDVLAKFWDE

SEQ ID NO: 7 - protein, 369 aa, Herpes simplex virus-2
MSQWGPRAILVQTDSTNRNADGDWQAAVAIRGGGVVQLNMVNKRAVDFTPAECGDSEWAVGRVSLGLRMAMPRDFCAIIHAPAVSGPGPHVMLGLVDSGYRGTVLAVVVAPNGTRGFAPGALRVDVTFLDIRATPPTLTEPSSLHRFPQLAPSPLAGLREDPWLDGALATAGGAVALPARRRGGSLVYAGELTQVTTEHGDCVHEAPAFLPKREEDAGFDILIHRAVTVPANGATVIQPSLRVLRAADGPEACYVLGRSSLNARGLLVMPTRWPSGHACAFVVCNLTGVPVTLQAGSKVAQLLVAGTHALPWIPPDNIHEDGAFRAYPRGVPDATATPRDPPILVFTNEFDADAPPSKRGAGGFGSTGI